European Patent Specification EP 4 196 595 B1, published March 12, 2025. Title: METHOD FOR THE TREATMENT OF WWOX ASSOCIATED DISEASES. Applicant: Yissum Research Development Company of the Hebrew University of Jerusalem Ltd. Aqeilan, Rami Repudi, Srinivas. The sequence listing filed with the application follows.

SEQUENCE LISTING (5 sequences)

SEQ ID NO: 1 - DNA, 1245 bp, Homo sapiens
atggcagcgctgcgctacgcggggctggacgacacggacagtgaggacgagctgcctccgggctgggaggagagaaccaccaaggacggctgggtttactacgccaatcacaccgaggagaagactcagtgggaacatccaaaaactggaaaaagaaaacgagtggcaggagatttgccatacggatgggaacaagaaactgatgagaacggacaagtgttttttgttgaccatataaataaaagaaccacctacttggacccaagactggcgtttactgtggatgataatccgaccaagccaaccacccggcaaagatacgacggcagcaccactgccatggaaattctccagggccgggatttcactggcaaagtggttgtggtcactggagctaattcaggaatagggttcgaaaccgccaagtcttttgccctccatggtgcacatgtgatcttggcctgcaggaacatggcaagggcgagtgaagcagtgtcacgcattttagaagaatggcataaagccaaggtagaagcaatgaccctggacctcgctctgctccgtagcgtgcagcattttgctgaagcattcaaggccaagaatgtgcctcttcatgtgcttgtgtgcaacgcagcaacttttgctctaccctggagtctcaccaaagatggcctggagaccacctttcaagtgaatcatctggggcacttctaccttgtccagctcctccaggatgttttgtgccgctcagctcctgcccgtgtcattgtggtctcctcagagtcccatcgatttacagatattaacgactccttgggaaaactggacttcagtcgcctctctccaacaaaaaacgactattgggcgatgctggcttataacaggtccaagctctgcaacatcctcttctccaacgagctgcaccgtcgcctctccccacgcggggtcacgtcgaacgcagtgcatcctggaaatatgatgtactccaacattcatcgcagctggtgggtgtacacactgctgtttaccttggcgaggcctttcaccaagtccatgcaacagggagctgccaccaccgtgtactgtgctgctgtcccagaactggagggtctgggagggatgtacttcaacaactgctgccgctgcatgccctcaccagaagctcagagcgaagagacggcccggaccctgtgggcgctcagcgagaggctgatccaagaacggcttggcagccagtccggctaa

SEQ ID NO: 2 - protein, 414 aa, Homo sapiens
MAALRYAGLDDTDSEDELPPGWEERTTKDGWVYYANHTEEKTQWEHPKTGKRKRVAGDLPYGWEQETDENGQVFFVDHINKRTTYLDPRLAFTVDDNPTKPTTRQRYDGSTTAMEILQGRDFTGKVVVVTGANSGIGFETAKSFALHGAHVILACRNMARASEAVSRILEEWHKAKVEAMTLDLALLRSVQHFAEAFKAKNVPLHVLVCNAATFALPWSLTKDGLETTFQVNHLGHFYLVQLLQDVLCRSAPARVIVVSSESHRFTDINDSLGKLDFSRLSPTKNDYWAMLAYNRSKLCNILFSNELHRRLSPRGVTSNAVHPGNMMYSNIHRSWWVYTLLFTLARPFTKSMQQGAATTVYCAAVPELEGLGGMYFNNCCRCMPSPEAQSEETARTLWALSERLIQERLGSQSG

SEQ ID NO: 3 - DNA, 2241 bp, Homo sapiens
gcagtgcgcaggcgtgagcggtcgggccccgacgcgcgcgggtctcgtttggagcgggagtgagttcctgagcgagtggacccggcagcgggcgataggggggccaggtgcctccacagtcagccatggcagcgctgcgctacgcggggctggacgacacggacagtgaggacgagctgcctccgggctgggaggagagaaccaccaaggacggctgggtttactacgccaatcacaccgaggagaagactcagtgggaacatccaaaaactggaaaaagaaaacgagtggcaggagatttgccatacggatgggaacaagaaactgatgagaacggacaagtgttttttgttgaccatataaataaaagaaccacctacttggacccaagactggcgtttactgtggatgataatccgaccaagccaaccacccggcaaagatacgacggcagcaccactgccatggaaattctccagggccgggatttcactggcaaagtggttgtggtcactggagctaattcaggaatagggttcgaaaccgccaagtcttttgccctccatggtgcacatgtgatcttggcctgcaggaacatggcaagggcgagtgaagcagtgtcacgcattttagaagaatggcataaagccaaggtagaagcaatgaccctggacctcgctctgctccgtagcgtgcagcattttgctgaagcattcaaggccaagaatgtgcctcttcatgtgcttgtgtgcaacgcagcaacttttgctctaccctggagtctcaccaaagatggcctggagaccacctttcaagtgaatcatctggggcacttctaccttgtccagctcctccaggatgttttgtgccgctcagctcctgcccgtgtcattgtggtctcctcagagtcccatcgatttacagatattaacgactccttgggaaaactggacttcagtcgcctctctccaacaaaaaacgactattgggcgatgctggcttataacaggtccaagctctgcaacatcctcttctccaacgagctgcaccgtcgcctctccccacgcggggtcacgtcgaacgcagtgcatcctggaaatatgatgtactccaacattcatcgcagctggtgggtgtacacactgctgtttaccttggcgaggcctttcaccaagtccatgcaacagggagctgccaccaccgtgtactgtgctgctgtcccagaactggagggtctgggagggatgtacttcaacaactgctgccgctgcatgccctcaccagaagctcagagcgaagagacggcccggaccctgtgggcgctcagcgagaggctgatccaagaacggcttggcagccagtccggctaagtggagctcagagcggatgggcacacacacccgccctgtgtgtgtcccctcacgcaagtgccagggctgggccccttccaaatgtccctccaacacagatccgcaagagtaaaggaaataagagcagtcacaacagagtgaaaaatcttaagtaccaatgggaagcagggaattcctggggtaaagtatcacttttctggggctgggctaggcataggtctctttgctttctggtggtggcctgtttgaaagtaaaaacctgcttggtgtgtaggttccgtatctccctggagaagcaccagcaattctctttcttttactgttatagaatagcctgaggtcccctcgtcccatccagctaccaccacggccaccactgcagccgggggctggccttctcctacttagggaagaaaaagcaagtgttcactgctccttgctgcattgatccaggagataattgtttcattcatcctgaccaagactgagccagcttagcaactgctggggagacaaatctcagaaccttgtcccagccagtgaggatgacagtgacacccagagggagtagaatacgcagaactaccaggtggcaaagtacttgtcatagactcctttgctaatgctatgcaaaaaattctttagagattataacaaatttttcaaatcattccttagataccttgaaaggcaggaagggaagcgtatatacttaagaatacacaggatattttggggggcagagaataaaacgttagttaatccctttgtctgtcaatcacagtctcagttctcttgctttcacattgtacttaaacctcctgctgtgcctcgcatcctatgcttaataaaagaacatgcttgaatatca

SEQ ID NO: 4 - DNA, 572 bp, Homo sapiens
actacaaaccgagtatctgcagagggccctgcgtatgagtgcaagtgggttttaggaccaggatgaggcggggtgggggtgcctacctgacgaccgaccccgacccactggacaagcacccaacccccattccccaaattgcgcatcccctatcagagagggggaggggaaacaggatgcggcgaggcgcgtgcgcactgccagcttcagcaccgcggacagtgccttcgcccccgcctggcggcgcgcgccaccgccgcctcagcactgaaggcgcgctgacgtcactcgccggtcccccgcaaactccccttcccggccaccttggtcgcgtccgcgccgccgccggcccagccggaccgcaccacgcgaggcgcgagataggggggcacgggcgcgaccatctgcgctgcggcgccggcgactcagcgctgcctcagtctgcggtgggcagcggaggagtcgtgtcgtgcctgagagcgcagctgtgctcctgggcaccgcgcagtccgcccccgcggctcctggccagaccacccctaggaccccctgccccaagtcgcagccttcga

SEQ ID NO: 5 - DNA, 6284 bp, Homo sapiens
cctgcaggcagctgcgcgctcgctcgctcactgaggccgcccgggcaaagcccgggcgtcgggcgacctttggtcgcccggcctcagtgagcgagcgagcgcgcagagagggagtggccaactccatcactaggggttcctgcggcaattcagtcgataactataacggtcctaaggtagcgatttaaatacgcgctctcttaaggtagccccgggacgcgtcaattgactacaaaccgagtatctgcagagggccctgcgtatgagtgcaagtgggttttaggaccaggatgaggcggggtgggggtgcctacctgacgaccgaccccgacccactggacaagcacccaacccccattccccaaattgcgcatcccctatcagagagggggaggggaaacaggatgcggcgaggcgcgtgcgcactgccagcttcagcaccgcggacagtgccttcgcccccgcctggcggcgcgcgccaccgccgcctcagcactgaaggcgcgctgacgtcactcgccggtcccccgcaaactccccttcccggccaccttggtcgcgtccgcgccgccgccggcccagccggaccgcaccacgcgaggcgcgagataggggggcacgggcgcgaccatctgcgctgcggcgccggcgactcagcgctgcctcagtctgcggtgggcagcggaggagtcgtgtcgtgcctgagagcgcagctgtgctcctgggcaccgcgcagtccgcccccgcggctcctggccagaccacccctaggaccccctgccccaagtcgcagccttcgagctagcgtttaaacttaagcttggtaccggccgctgcggccctcgagcaagctggctagttaagctatcaacaagtttgtacaaaaaagcaggctttaaaggaaccaattcagtcgagaattcgtcgactggatccggtaccgaggagatctgccgccgcgatcgccgcagtgcgcaggcgtgagcggtcgggccccgacgcgcgcgggtctcgtttggagcgggagtgagttcctgagcgagtggacccggcagcgggcgataggggggccaggtgcctccacagtcagccatggcagcgctgcgctacgcggggctggacgacacggacagtgaggacgagctgcctccgggctgggaggagagaaccaccaaggacggctgggtttactacgccaatcacaccgaggagaagactcagtgggaacatccaaaaactggaaaaagaaaacgagtggcaggagatttgccatacggatgggaacaagaaactgatgagaacggacaagtgttttttgttgaccatataaataaaagaaccacctacttggacccaagactggcgtttactgtggatgataatccgaccaagccaaccacccggcaaagatacgacggcagcaccactgccatggaaattctccagggccgggatttcactggcaaagtggttgtggtcactggagctaattcaggaatagggttcgaaaccgccaagtcttttgccctccatggtgcacatgtgatcttggcctgcaggaacatggcaagggcgagtgaagcagtgtcacgcattttagaagaatggcataaagccaaggtagaagcaatgaccctggacctcgctctgctccgtagcgtgcagcattttgctgaagcattcaaggccaagaatgtgcctcttcatgtgcttgtgtgcaacgcagcaacttttgctctaccctggagtctcaccaaagatggcctggagaccacctttcaagtgaatcatctggggcacttctaccttgtccagctcctccaggatgttttgtgccgctcagctcctgcccgtgtcattgtggtctcctcagagtcccatcgatttacagatattaacgactccttgggaaaactggacttcagtcgcctctctccaacaaaaaacgactattgggcgatgctggcttataacaggtccaagctctgcaacatcctcttctccaacgagctgcaccgtcgcctctccccacgcggggtcacgtcgaacgcagtgcatcctggaaatatgatgtactccaacattcatcgcagctggtgggtgtacacactgctgtttaccttggcgaggcctttcaccaagtccatgcaacagggagctgccaccaccgtgtactgtgctgctgtcccagaactggagggtctgggagggatgtacttcaacaactgctgccgctgcatgccctcaccagaagctcagagcgaagagacggcccggaccctgtgggcgctcagcgagaggctgatccaagaacggcttggcagccagtccggctaagtggagctcagagcggatgggcacacacacccgccctgtgtgtgtcccctcacgcaagtgccagggctgggccccttccaaatgtccctccaacacagatccgcaagagtaaaggaaataagagcagtcacaacagagtgaaaaatcttaagtaccaatgggaagcagggaattcctggggtaaagtatcacttttctggggctgggctaggcataggtctctttgctttctggtggtggcctgtttgaaagtaaaaacctgcttggtgtgtaggttccgtatctccctggagaagcaccagcaattctctttcttttactgttatagaatagcctgaggtcccctcgtcccatccagctaccaccacggccaccactgcagccgggggctggccttctcctacttagggaagaaaaagcaagtgttcactgctccttgctgcattgatccaggagataattgtttcattcatcctgaccaagactgagccagcttagcaactgctggggagacaaatctcagaaccttgtcccagccagtgaggatgacagtgacacccagagggagtagaatacgcagaactaccaggtggcaaagtacttgtcatagactcctttgctaatgctatgcaaaaaattctttagagattataacaaatttttcaaatcattccttagataccttgaaaggcaggaagggaagcgtatatacttaagaatacacaggatattttggggggcagagaataaaacgttagttaatccctttgtctgtcaatcacagtctcagttctcttgctttcacattgtacttaaacctcctgctgtgcctcgcatcctatgcttaataaaagaacatgcttgaatatcattgagtttaaacccgctgatcagcctcgactgtgccttctagttgccagccatctgttgtttgcccctcccccgtgccttccttgaccctggaaggtgccactcccactgtcctttcctaataaaatgaggaaattgcatcgcattgtctgagtaggtgtcattctattctggggggtggggtggggcaggacagcaagggggaggattgggaagacaatagcaggcatgctggggatgcggtgggctctatggcttctgaggcggaaagaaccagatcctctcttaaggtagcatcgagatttaaattagggataacagggtaatggcgcgggccgcaggaacccctagtgatggagttggccactccctctctgcgcgctcgctcgctcactgaggccgggcgaccaaaggtcgcccgacgcccgggctttgcccgggcggcctcagtgagcgagcgagcgcgcagctgcctgcaggggcgcctgatgcggtattttctccttacgcatctgtgcggtatttcacaccgcatacgtcaaagcaaccatagtacgcgccctgtagcggcgcattaagcgcggcgggtgtggtggttacgcgcagcgtgaccgctacacttgccagcgccctagcgcccgctcctttcgctttcttcccttcctttctcgccacgttcgccggctttccccgtcaagctctaaatcgggggctccctttagggttccgatttagtgctttacggcacctcgaccccaaaaaacttgatttgggtgatggttcacgtagtgggccatcgccctgatagacggtttttcgccctttgacgttggagtccacgttctttaatagtggactcttgttccaaactggaacaacactcaaccctatctcgggctattcttttgatttataagggattttgccgatttcggcctattggttaaaaaatgagctgatttaacaaaaatttaacgcgaattttaacaaaatattaacgtttacaattttatggtgcactctcagtacaatctgctctgatgccgcatagttaagccagccccgacacccgccaacacccgctgacgcgccctgacgggcttgtctgctcccggcatccgcttacagacaagctgtgaccgtctccgggagctgcatgtgtcagaggttttcaccgtcatcaccgaaacgcgcgagacgaaagggcctcgtgatacgcctatttttataggttaatgtcatgataataatggtttcttagacgtcaggtggcacttttcggggaaatgtgcgcggaacccctatttgtttatttttctaaatacattcaaatatgtatccgctcatgagacaataaccctgataaatgcttcaataatattgaaaaaggaagagtatgagtattcaacatttccgtgtcgcccttattcccttttttgcggcattttgccttcctgtttttgctcacccagaaacgctggtgaaagtaaaagatgctgaagatcagttgggtgcacgagtgggttacatcgaactggatctcaacagcggtaagatccttgagagttttcgccccgaagaacgttttccaatgatgagcacttttaaagttctgctatgtggcgcggtattatcccgtattgacgccgggcaagagcaactcggtcgccgcatacactattctcagaatgacttggttgagtactcaccagtcacagaaaagcatcttacggatggcatgacagtaagagaattatgcagtgctgccataaccatgagtgataacactgcggccaacttacttctgacaacgatcggaggaccgaaggagctaaccgcttttttgcacaacatgggggatcatgtaactcgccttgatcgttgggaaccggagctgaatgaagccataccaaacgacgagcgtgacaccacgatgcctgtagcaatggcaacaacgttgcgcaaactattaactggcgaactacttactctagcttcccggcaacaattaatagactggatggaggcggataaagttgcaggaccacttctgcgctcggcccttccggctggctggtttattgctgataaatctggagccggtgagcgtgggtctcgcggtatcattgcagcactggggccagatggtaagccctcccgtatcgtagttatctacacgacggggagtcaggcaactatggatgaacgaaatagacagatcgctgagataggtgcctcactgattaagcattggtaactgtcagaccaagtttactcatatatactttagattgatttaaaacttcatttttaatttaaaaggatctaggtgaagatcctttttgataatctcatgaccaaaatcccttaacgtgagttttcgttccactgagcgtcagaccccgtagaaaagatcaaaggatcttcttgagatcctttttttctgcgcgtaatctgctgcttgcaaacaaaaaaaccaccgctaccagcggtggtttgtttgccggatcaagagctaccaactctttttccgaaggtaactggcttcagcagagcgcagataccaaatactgtccttctagtgtagccgtagttaggccaccacttcaagaactctgtagcaccgcctacatacctcgctctgctaatcctgttaccagtggctgctgccagtggcgataagtcgtgtcttaccgggttggactcaagacgatagttaccggataaggcgcagcggtcgggctgaacggggggttcgtgcacacagcccagcttggagcgaacgacctacaccgaactgagatacctacagcgtgagctatgagaaagcgccacgcttcccgaagggagaaaggcggacaggtatccggtaagcggcagggtcggaacaggagagcgcacgagggagcttccagggggaaacgcctggtatctttatagtcctgtcgggtttcgccacctctgacttgagcgtcgatttttgtgatgctcgtcaggggggcggagcctatggaaaaacgccagcaacgcggcctttttacggttcctggccttttgctggccttttgctcacatgt